European Patent Specification EP 3 925 997 B1, published July 17, 2024. Title: Biomass-Resource-Derived Polyester and Production Process Thereof. Applicant: Mitsubishi Chemical Corporation. The sequence listing filed with the application follows.

SEQUENCE LISTING (16 sequences)

SEQ ID NO: 1 - DNA, 34 bp, Artificial
  Source: /note = "Description of Artificial Sequence: primer"
cctttttaacccatcacatatacctgccgttcac

SEQ ID NO: 2 - DNA, 32 bp, Artificial
  Source: /note = "Description of Artificial Sequence: primer"
aaaggttaggaatacggttagccatttgcctg

SEQ ID NO: 3 - DNA, 21 bp, Artificial
  Source: /note = "Description of Artificial Sequence: primer"
gaggtctgcctcgtgaagaag

SEQ ID NO: 4 - DNA, 27 bp, Artificial
  Source: /note = "Description of Artificial Sequence: primer"
ctcattagaaaaactcatcgagcatca

SEQ ID NO: 5 - DNA, 20 bp, Artificial
  Source: /note = "Description of Artificial Sequence: primer"
cgatgaaagaaaccgtcggc

SEQ ID NO: 6 - DNA, 20 bp, Artificial
  Source: /note = "Description of Artificial Sequence: primer"
cgtcagaagaactgcttctg

SEQ ID NO: 7 - DNA, 23 bp, Artificial
  Source: /note = "Description of Artificial Sequence: primer"
agttgcatacgcatacgcactga

SEQ ID NO: 8 - DNA, 23 bp, Artificial
  Source: /note = "Description of Artificial Sequence: primer"
gagactgggactgcaacgtcttg

SEQ ID NO: 9 - DNA, 24 bp, Artificial
  Source: /note = "Description of Artificial Sequence: primer"
gatctttcagctgctcacacgtga

SEQ ID NO: 10 - DNA, 27 bp, Artificial
  Source: /note = "Description of Artificial Sequence: primer"
gatcttaggtcactaaaactaattcag

SEQ ID NO: 11 - DNA, 39 bp, Artificial
  Source: /note = "Description of Artificial Sequence: primer"
gatccaggaggcattaattaagcggccgcgggccctgca

SEQ ID NO: 12 - DNA, 31 bp, Artificial
  Source: /note = "Description of Artificial Sequence: primer"
gggcccgcggccgcttaattaatgcctcctg

SEQ ID NO: 13 - DNA, 43 bp, Artificial
  Source: /note = "Description of Artificial Sequence: primer"
accttaattaatgtcgactcacacatcttcaacgcttccagca

SEQ ID NO: 14 - DNA, 44 bp, Artificial
  Source: /note = "Description of Artificial Sequence: primer"
gttgggcccaggtttaggaaacgacgacgatcaagtcgccacct

SEQ ID NO: 15 - DNA, 3423 bp, Brevibacterium flavum
  CDS (1)..(3420)
atgtcgactcacacatcttcaacgcttccagcattcaaaaagatcttggtagcaaaccgcggcgaaatcgcggtccgtgctttccgtgcagcactcgaaaccggtgcagccacggtagctatttacccccgtgaagatcggggatcattccaccgctcttttgcttctgaagctgtccgcattggtactgaaggctcaccagtcaaggcgtacctggacatcgatgaaattatcggtgcagctaaaaaagttaaagcagatgctatttacccgggatatggcttcctgtctgaaaatgcccagcttgcccgcgagtgcgcggaaaacggcattacttttattggcccaaccccagaggttcttgatctcaccggtgataagtctcgtgcggtaaccgccgcgaagaaggctggtctgccagttttggcggaatccaccccgagcaaaaacatcgatgacatcgttaaaagcgctgaaggccagacttaccccatctttgtaaaggcagttgccggtggtggcggacgcggtatgcgctttgtttcttcacctgatgagcttcgcaaattggcaacagaagcatctcgtgaagctgaagcggcattcggcgacggttcggtatatgtcgagcgtgctgtgattaacccccagcacattgaagtgcagatccttggcgatcgcactggagaagttgtacacctttatgaacgtgactgctcactgcagcgtcgtcaccaaaaagttgtcgaaattgcgccagcacagcatttggatccagaactgcgtgatcgcatttgtgcggatgcagtaaagttctgccgctccattggttaccagggcgcgggaactgtggaattcttggtcgatgaaaagggcaaccacgttttcatcgaaatgaacccacgtatccaggttgagcacaccgtgactgaagaagtcaccgaggtggacctggtgaaggcgcagatgcgcttggctgctggtgcaaccttgaaggaattgggtctgacccaagataagatcaagacccacggtgcggcactgcagtgccgcatcaccacggaagatccaaacaacggcttccgcccagataccggaactatcaccgcgtaccgctcaccaggcggagctggcgttcgtcttgacggtgcagctcagctcggtggcgaaatcaccgcacactttgactccatgctggtgaaaatgacctgccgtggttccgattttgaaactgctgttgctcgtgcacagcgcgcgttggctgagttcaccgtgtctggtgttgcaaccaacattggtttcttgcgtgcgttgctgcgtgaagaggactttacttccaagcgcatcgccaccggatttatcggcgatcacccacacctccttcaggctccacctgcggatgatgagcagggacgcatcctggattacttggcagatgtcaccgtgaacaagcctcatggtgtgcgtccaaaggatgttgcagcaccaatcgataagctgcccaacatcaaggatctgccactgccacgcggttcccgtgaccgcctgaagcagcttggaccagcagcgtttgcccgcgatctccgtgagcaggacgcactggcagttactgataccaccttccgcgatgcacaccagtctttgcttgcgacccgagtccgctcattcgcactgaagcctgcggcagaggccgtcgcaaagctgactcctgagcttttgtccgtggaggcctggggcggtgcgacctacgatgtggcgatgcgtttcctctttgaggatccgtgggacaggctcgacgagctgcgcgaggcgatgccgaatgtgaacattcagatgctgcttcgcggccgcaacaccgtgggatacaccccatacccagactccgtctgtcgcgcgtttgttaaggaagctgccacctccggcgtggacatcttccgcatcttcgacgcgcttaacgacgtctcccagatgcgtccagcaatcgacgcagtcctggagaccaacaccgcggtcgctgaagtggctatggcttattctggtgatctttccgatccgaatgaaaagctctacaccctggattactacctgaagatggcagaggagatcgtcaagtctggcgctcacattctggctattaaggatatggctggtctgcttcgcccagctgcagccaccaagctggtcaccgcactgcgccgtgaatttgatctgccagtgcacgtgcacacccacgacactgcgggtggccagctggcaacctactttgctgcagctcaagctggtgcagatgctgttgacggtgcttccgcaccactgtctggcaccacctcccagccatccctgtctgccattgttgctgcattcgcgcacacccgtcgcgataccggtttgagcctcgaggctgtttctgacctcgagccatactgggaagcagtgcgcggactgtacctgccatttgagtctggaaccccaggcccaaccggtcgcgtctaccgccacgaaatcccaggcggacagctgtccaacctgcgtgcacaggccaccgcactgggccttgcggatcgtttcgaactcatcgaagacaactacgcggcagttaatgagatgctgggacgcccaaccaaggtcaccccatcctccaaggttgttggcgacctcgcactccacctcgttggtgcgggtgtggatccagcagactttgctgcagatccacaaaagtacgacatcccagactctgtcatcgcgttcctgcgcggcgagcttggtaaccctccaggtggctggccagagccactgcgcacccgcgcactggaaggccgctccgaaggcaaggcacctctgacggaagttcctgaggaagagcaggcgcacctcgacgctgatgattccaaggaacgtcgcaacagcctcaaccgcctgctgttcccgaagccaaccgaagagttcctcgagcaccgtcgccgcttcggcaacacctctgcgctggatgatcgtgaattcttctacggcctggtcgaaggccgcgagactttgatccgcctgccagatgtgcgcaccccactgcttgttcgcctggatgcgatctccgagccagacgataagggtatgcgcaatgttgtggccaacgtcaacggccagatccgcccaatgcgtgtgcgtgaccgctccgttgagtctgtcaccgcaaccgcagaaaaggcagattcctccaacaagggccatgttgctgcaccattcgctggtgttgtcactgtgactgttgctgaaggtgatgaggtcaaggctggagatgcagtcgcaatcatcgaggctatgaagatggaagcaacaatcactgcttctgttgacggcaaaatcgatcgcgttgtggttcctgctgcaacgaaggtggaaggtggcgacttgatcgtcgtcgtttcctaa

SEQ ID NO: 16 - protein, 1140 aa, Brevibacterium flavum
MSTHTSSTLPAFKKILVANRGEIAVRAFRAALETGAATVAIYPREDRGSFHRSFASEAVRIGTEGSPVKAYLDIDEIIGAAKKVKADAIYPGYGFLSENAQLARECAENGITFIGPTPEVLDLTGDKSRAVTAAKKAGLPVLAESTPSKNIDDIVKSAEGQTYPIFVKAVAGGGGRGMRFVSSPDELRKLATEASREAEAAFGDGSVYVERAVINPQHIEVQILGDRTGEVVHLYERDCSLQRRHQKVVEIAPAQHLDPELRDRICADAVKFCRSIGYQGAGTVEFLVDEKGNHVFIEMNPRIQVEHTVTEEVTEVDLVKAQMRLAAGATLKELGLTQDKIKTHGAALQCRITTEDPNNGFRPDTGTITAYRSPGGAGVRLDGAAQLGGEITAHFDSMLVKMTCRGSDFETAVARAQRALAEFTVSGVATNIGFLRALLREEDFTSKRIATGFIGDHPHLLQAPPADDEQGRILDYLADVTVNKPHGVRPKDVAAPIDKLPNIKDLPLPRGSRDRLKQLGPAAFARDLREQDALAVTDTTFRDAHQSLLATRVRSFALKPAAEAVAKLTPELLSVEAWGGATYDVAMRFLFEDPWDRLDELREAMPNVNIQMLLRGRNTVGYTPYPDSVCRAFVKEAATSGVDIFRIFDALNDVSQMRPAIDAVLETNTAVAEVAMAYSGDLSDPNEKLYTLDYYLKMAEEIVKSGAHILAIKDMAGLLRPAAATKLVTALRREFDLPVHVHTHDTAGGQLATYFAAAQAGADAVDGASAPLSGTTSQPSLSAIVAAFAHTRRDTGLSLEAVSDLEPYWEAVRGLYLPFESGTPGPTGRVYRHEIPGGQLSNLRAQATALGLADRFELIEDNYAAVNEMLGRPTKVTPSSKVVGDLALHLVGAGVDPADFAADPQKYDIPDSVIAFLRGELGNPPGGWPEPLRTRALEGRSEGKAPLTEVPEEEQAHLDADDSKERRNSLNRLLFPKPTEEFLEHRRRFGNTSALDDREFFYGLVEGRETLIRLPDVRTPLLVRLDAISEPDDKGMRNVVANVNGQIRPMRVRDRSVESVTATAEKADSSNKGHVAAPFAGVVTVTVAEGDEVKAGDAVAIIEAMKMEATITASVDGKIDRVVVPAATKVEGGDLIVVVS